European Patent Specification EP 3 430 045 B1, published August 23, 2023. Title: Anti-TNF-alpha antibodies and functional fragments thereof. Applicant: Tillotts Pharma AG. The sequence listing filed with the application follows.

SEQUENCE LISTING (37 sequences)

SEQ ID NO: 1 - protein, 11 aa, Artificial Sequence
  Generic CDR L1
  MISC_FEATURE (7)..(7): Xaa is Ser or Gly
  MISC_FEATURE (8)..(8): Xaa is Ser or Asn
  MISC_FEATURE (11)..(11): Xaa is Ala or Ser
QASQSIXXYLX

SEQ ID NO: 2 - protein, 7 aa, Artificial Sequence
  Generic CDR L2
  MISC_FEATURE (1)..(1): Xaa is Arg, Gln or Lys
XASTLAS

SEQ ID NO: 3 - protein, 13 aa, Artificial Sequence
  Generic CDR L3
  misc_feature (2)..(2): Xaa can be any naturally occurring amino acid
QXTYYEPSYVFRA

SEQ ID NO: 4 - protein, 11 aa, Artificial Sequence
  Generic CDR H1
  MISC_FEATURE (1)..(1): Xaa is Arg or Gly
XIDFSAGYDMC

SEQ ID NO: 5 - protein, 17 aa, Artificial Sequence
  Generic CDR H2
  MISC_FEATURE (6)..(6): Xaa is Arg, Asn or Ser
  MISC_FEATURE (7)..(7): Xaa is Asp or Glu
  MISC_FEATURE (8)..(8): Xaa is Asn, Asp or Glu
  MISC_FEATURE (9)..(9): Xaa is Ser or Thr
CIDSRXXXXDYASWAKG

SEQ ID NO: 6 - protein, 14 aa, Artificial Sequence
  CDR H3 of clones 17-22-B03, 16-12-E09, 16-13-E01, 16-15-E11, 16-17-C08, 16-17-G01, 17-18-D10 and 17-22-B01
GGYGGDGVDGAFDP

SEQ ID NO: 7 - protein, 11 aa, Artificial Sequence
  CDR L1 of clones 17-22-B03, 16-12-E09, 16-13-E01, 16-15-E11 and 17-18-D10
QASQSISSYLA

SEQ ID NO: 8 - protein, 7 aa, Artificial Sequence
  CDR L2 of clones 17-22-B03, 16-12-E09, 16-15-E11, 16-17-C08, 16-17-G01 and 17-18-D10
KASTLAS

SEQ ID NO: 9 - protein, 13 aa, Artificial Sequence
  CDR L3 of clones 17-22-B03, 16-12-E09, 16-13-E01, 16-15-E11, 16-17-C08, 16-17-G01, 17-18-D10 and 17-22-B01
QCTYYEPSYVFRA

SEQ ID NO: 10 - protein, 11 aa, Artificial Sequence
  CDR H1 of clones 17-22-B03, 16-12-E09, 16-13-E01, 16-15-E11, 16-17-C08, 17-18-D10 and 17-22-B01
GIDFSAGYDMC

SEQ ID NO: 11 - protein, 17 aa, Artificial Sequence
  CDR H2 of clones 17-22-B03 and 16-17-C08
CIDSRREESDYASWAKG

SEQ ID NO: 12 - protein, 17 aa, Artificial Sequence
  CDR H2 of clone 16-12-E09
CIDSRSDNTDYASWAKG

SEQ ID NO: 13 - protein, 7 aa, Artificial Sequence
  CDR L2 of clone 16-13-E01
QASTLAS

SEQ ID NO: 14 - protein, 17 aa, Artificial Sequence
  CDR H2 of clones 16-13-E01 and 17-18-D10
CIDSRREDSDYASWAKG

SEQ ID NO: 15 - protein, 17 aa, Artificial Sequence
  CDR H2 of clones 16-15-E11, 16-17-G01 and 17-22-B01
CIDSRNDNTDYASWAKG

SEQ ID NO: 16 - protein, 11 aa, Artificial Sequence
  CDR L1 of clone 16-17-C08
QASQSIGSYLA

SEQ ID NO: 17 - protein, 11 aa, Artificial Sequence
  CDR L1 of clone 16-17-G01
QASQSISNYLA

SEQ ID NO: 18 - protein, 11 aa, Artificial Sequence
  CDR H1 of clone 16-17-G01
RIDFSAGYDMC

SEQ ID NO: 19 - protein, 11 aa, Artificial Sequence
  CDR L1 of clone 17-22-B01
QASQSISSYLS

SEQ ID NO: 20 - protein, 7 aa, Artificial Sequence
  CDR L2 of clone 17-22-B01
RASTLAS

SEQ ID NO: 21 - protein, 124 aa, Artificial Sequence
  VH of humanized scFv of clones 17-22-B03-sc02, 17-22-B03-sc08, 17-22-B03-sc12
EVQLVESGGGLVQPGGSLRLSCKASGIDFSAGYDMCWVRQAPGKGLEWIACIDSRREESDYASWAKGRFTISKDSSKNTVYLQMNSLRAEDTAVYYCARGGYGGDGVDGAFDPWGQGTLVTVSS

SEQ ID NO: 22 - protein, 112 aa, Artificial Sequence
  VL of humanized scFv of clone 17-22-B03-sc02
DIQMTQSPSSLSASVGDRVTIKCQASQSISSYLAWYQQKPGKAPKLLIYKASTLASGVPSRFSGSGSGTEFTLTISDLEPADFATYYCQCTYYEPSYVFRAFGGGTKLTVLG

SEQ ID NO: 23 - protein, 112 aa, Artificial Sequence
  VL of humanized scFv of clone 17-22-B03-sc08
DIQMTQSPSSLSASVGDRVTITCQASQSISSYLAWYQQKPGKAPKLLIYKASTLASGVPSRFSGSGSGTDFTLTISSLQPEDFATYYCQCTYYEPSYVFRAFGGGTKLTVLG

SEQ ID NO: 24 - protein, 112 aa, Artificial Sequence
  VL of humanized scFv of clone 17-22-B03-sc12
DIQMTQSPSSLSASVGDRVTITCQASQSISSYLAWYQQKPGKAPKLLIYKASTLASGVPSRFSGSGSGTDFTLTISSLQPEDFATYYCQSTYYEPSYVFRAFGGGTKLTVLG

SEQ ID NO: 25 - protein, 257 aa, Artificial Sequence
  Humanized scFv of clone 17-22-B03-sc02
MDIQMTQSPSSLSASVGDRVTIKCQASQSISSYLAWYQQKPGKAPKLLIYKASTLASGVPSRFSGSGSGTEFTLTISDLEPADFATYYCQCTYYEPSYVFRAFGGGTKLTVLGGGGGSGGGGSGGGGSGGGGSEVQLVESGGGLVQPGGSLRLSCKASGIDFSAGYDMCWVRQAPGKGLEWIACIDSRREESDYASWAKGRFTISKDSSKNTVYLQMNSLRAEDTAVYYCARGGYGGDGVDGAFDPWGQGTLVTVSS

SEQ ID NO: 26 - protein, 257 aa, Artificial Sequence
  Humanized scFv of clone 17-22-B03-sc08
MDIQMTQSPSSLSASVGDRVTITCQASQSISSYLAWYQQKPGKAPKLLIYKASTLASGVPSRFSGSGSGTDFTLTISSLQPEDFATYYCQCTYYEPSYVFRAFGGGTKLTVLGGGGGSGGGGSGGGGSGGGGSEVQLVESGGGLVQPGGSLRLSCKASGIDFSAGYDMCWVRQAPGKGLEWIACIDSRREESDYASWAKGRFTISKDSSKNTVYLQMNSLRAEDTAVYYCARGGYGGDGVDGAFDPWGQGTLVTVSS

SEQ ID NO: 27 - protein, 257 aa, Artificial Sequence
  Humanized scFv of clone 17-22-B03-sc12
MDIQMTQSPSSLSASVGDRVTITCQASQSISSYLAWYQQKPGKAPKLLIYKASTLASGVPSRFSGSGSGTDFTLTISSLQPEDFATYYCQSTYYEPSYVFRAFGGGTKLTVLGGGGGSGGGGSGGGGSGGGGSEVQLVESGGGLVQPGGSLRLSCKASGIDFSAGYDMCWVRQAPGKGLEWIACIDSRREESDYASWAKGRFTISKDSSKNTVYLQMNSLRAEDTAVYYCARGGYGGDGVDGAFDPWGQGTLVTVSS

SEQ ID NO: 28 - protein, 13 aa, Artificial Sequence
  Generic CDR L3 where Cys2 (Xaa) is limited to Arg, His, Pro, Phe, Gln, Gly or Tyr
  MISC_FEATURE (2)..(2): Xaa is Arg, His, Pro, Phe, Gln, Gly or Tyr
QXTYYEPSYVFRA

SEQ ID NO: 29 - protein, 20 aa, Artificial Sequence
  Linker sequence in scFv
GGGGSGGGGSGGGGSGGGGS

SEQ ID NO: 30 - protein, 5 aa, Artificial Sequence
  Linker sequence in diabody
GGGGS

SEQ ID NO: 31 - protein, 23 aa, Artificial Sequence
  Vk1 consensus sequence of framework I (Kabat positions 1-23)
DIQMTQSPSSLSASVGDRVTITC

SEQ ID NO: 32 - protein, 15 aa, Artificial Sequence
  Vk1 consensus sequence of framework II (Kabat positions 35-49)
WYQQKPGKAPKLLIY

SEQ ID NO: 33 - protein, 32 aa, Artificial Sequence
  Vk1 consensus sequence of framework III (Kabat positions 57-88)
GVPSRFSGSGSGTDFTLTISSLQPEDFATYYC

SEQ ID NO: 34 - protein, 10 aa, Artificial Sequence
  V lamda germline-based sequence of framework IV
FGTGTKVTVL

SEQ ID NO: 35 - protein, 10 aa, Artificial Sequence
  V lamda germline-based sequence of framework IV
FGGGTKLTVL

SEQ ID NO: 36 - protein, 10 aa, Artificial Sequence
  V lamda germline-based sequence of framework IV
FGGGTQLIIL

SEQ ID NO: 37 - protein, 10 aa, Artificial Sequence
  V lamda germline-based sequence of framework IV
FGSGTKVTVL